European Patent Specification EP 3 710 013 B1, published July 30, 2025. Title: METHODS AND COMPOSITIONS FOR NON-MYELOABLATIVE BONE MARROW RECONSTITUTION. Applicant: Weird Science LLC Gumrukcu, Serhat. The sequence listing filed with the application follows.

SEQUENCE LISTING (19 sequences)

SEQ ID NO: 1 - DNA, 1503 bp, Artificial Sequence
  hALDH1-cDNA
atgtcatcctcaggcacgccagacttacctgtcctactcaccgatttgaagattcaatatactaagatcttcataaacaatgaatggcatgattcagtgagtggcaagaaatttcctgtctttaatcctgcaactgaggaggagctctgccaggtagaagaaggagataaggaggatgttgacaaggcagtgaaggccgcaagacaggcttttcagattggatccccgtggcgtactatggatgcttccgagagggggcgactattatacaagttggctgatttaatcgaaagagatcgtctgctgctggcgacaatggagtcaatgaatggtggaaaactctattccaatgcatatctgaatgatttagcaggctgcatcaaaacattgcgctactgtgcaggttgggctgacaagatccagggccgtacaataccaattgatggaaatttttttacatatacaagacatgaacctattggtgtatgtggccaaatcattccttggaatttcccgttggttatgctcatttggaagatagggcctgcactgagctgtggaaacacagtggttgtcaaaccagcagagcaaactcctctcactgctctccacgtggcatctttaataaaagaggcagggtttcctcctggagtagtgaatattgttcctggttatgggcctacagcaggggcagccatttcttctcacatggatatagacaaagtagccttcacaggatcaacagaggttggcaagttgatcaaagaagctgccgggaaaagcaatctgaagagggtgaccctggagcttggaggaaagagcccttgcattgtgttagctgatgccgacttggacaatgctgttgaatttgcacaccatggggtattctaccaccagggccagtgttgtatagccgcatccaggatttttgtggaagaatcaatttatgatgagtttgttcgaaggagtgttgagcgggctaagaagtatatccttggaaatcctctgaccccaggagtcactcaaggccctcagattgacaaggaacaatatgataaaatacttgacctcattgagagtgggaagaaagaaggggccaaactggaatgtggaggaggcccgtgggggaataaaggctactttgtccagcccacagtgttctctaatgttacagatgagatgcgcattgccaaagaggagatttttggaccagtgcagcaaatcatgaagtttaaatctttagatgacgtgatcaaaagagcaaacaatactttctatggcttatcagcaggagtgtttaccaaagacattgataaagccataacaatctcctctgctctgcaggcaggaacagtgtgggtgaattgctatggcgtggtaagtgcccagtgcccctttggtggattcaagatgtctggaaatggaagagaactgggagagtacggtttccatgaatatacagaggtcaaaacagtcacagtgaaaatctctcagaagaactca

SEQ ID NO: 2 - DNA, 10781 bp, Artificial Sequence
  pLV-Puro-EF1A-hALDH1A1:T2A:EGFP
aatgtagtcttatgcaatactcttgtagtcttgcaacatggtaacgatgagttagcaacatgccttacaaggagagaaaaagcaccgtgcatgccgattggtggaagtaaggtggtacgatcgtgccttattaggaaggcaacagacgggtctgacatggattggacgaaccactgaattgccgcattgcagagatattgtatttaagtgcctagctcgatacataaacgggtctctctggttagaccagatctgagcctgggagctctctggctaactagggaacccactgcttaagcctcaataaagcttgccttgagtgcttcaagtagtgtgtgcccgtctgttgtgtgactctggtaactagagatccctcagacccttttagtcagtgtggaaaatctctagcagtggcgcccgaacagggacttgaaagcgaaagggaaaccagaggagctctctcgacgcaggactcggcttgctgaagcgcgcacggcaagaggcgaggggcggcgactggtgagtacgccaaaaattttgactagcggaggctagaaggagagagatgggtgcgagagcgtcagtattaagcgggggagaattagatcgcgatgggaaaaaattcggttaaggccagggggaaagaaaaaatataaattaaaacatatagtatgggcaagcagggagctagaacgattcgcagttaatcctggcctgttagaaacatcagaaggctgtagacaaatactgggacagctacaaccatcccttcagacaggatcagaagaacttagatcattatataatacagtagcaaccctctattgtgtgcatcaaaggatagagataaaagacaccaaggaagctttagacaagatagaggaagagcaaaacaaaagtaagaccaccgcacagcaagcggccgctgatcttcagacctggaggaggagatatgagggacaattggagaagtgaattatataaatataaagtagtaaaaattgaaccattaggagtagcacccaccaaggcaaagagaagagtggtgcagagagaaaaaagagcagtgggaataggagctttgttccttgggttcttgggagcagcaggaagcactatgggcgcagcgtcaatgacgctgacggtacaggccagacaattattgtctggtatagtgcagcagcagaacaatttgctgagggctattgaggcgcaacagcatctgttgcaactcacagtctggggcatcaagcagctccaggcaagaatcctggctgtggaaagatacctaaaggatcaacagctcctggggatttggggttgctctggaaaactcatttgcaccactgctgtgccttggaatgctagttggagtaataaatctctggaacagatttggaatcacacgacctggatggagtgggacagagaaattaacaattacacaagcttaatacactccttaattgaagaatcgcaaaaccagcaagaaaagaatgaacaagaattattggaattagataaatgggcaagtttgtggaattggtttaacataacaaattggctgtggtatataaaattattcataatgatagtaggaggcttggtaggtttaagaatagtttttgctgtactttctatagtgaatagagttaggcagggatattcaccattatcgtttcagacccacctcccaaccccgaggggacccgacaggcccgaaggaatagaagaagaaggtggagagagagacagagacagatccattcgattagtgaacggatctcgacggtatcgctagcttttaaaagaaaaggggggattggggggtacagtgcaggggaaagaatagtagacataatagcaacagacatacaaactaaagaattacaaaaacaaattacaaaaattcaaaattttactagtgattatcggatcaactttgtatagaaaagttgggctccggtgcccgtcagtgggcagagcgcacatcgcccacagtccccgagaagttggggggaggggtcggcaattgaaccggtgcctagagaaggtggcgcggggtaaactgggaaagtgatgtcgtgtactggctccgcctttttcccgagggtgggggagaaccgtatataagtgcagtagtcgccgtgaacgttctttttcgcaacgggtttgccgccagaacacaggtaagtgccgtgtgtggttcccgcgggcctggcctctttacgggttatggcccttgcgtgccttgaattacttccacctggctgcagtacgtgattcttgatcccgagcttcgggttggaagtgggtgggagagttcgaggccttgcgcttaaggagccccttcgcctcgtgcttgagttgaggcctggcctgggcgctggggccgccgcgtgcgaatctggtggcaccttcgcgcctgtctcgctgctttcgataagtctctagccatttaaaatttttgatgacctgctgcgacgctttttttctggcaagatagtcttgtaaatgcgggccaagatctgcacactggtatttcggtttttggggccgcgggcggcgacggggcccgtgcgtcccagcgcacatgttcggcgaggcggggcctgcgagcgcggccaccgagaatcggacgggggtagtctcaagctggccggcctgctctggtgcctggtctcgcgccgccgtgtatcgccccgccctgggcggcaaggctggcccggtcggcaccagttgcgtgagcggaaagatggccgcttcccggccctgctgcagggagctcaaaatggaggacgcggcgctcgggagagcgggcgggtgagtcacccacacaaaggaaaagggcctttccgtcctcagccgtcgcttcatgtgactccacggagtaccgggcgccgtccaggcacctcgattagttctcgagcttttggagtacgtcgtctttaggttggggggaggggttttatgcgatggagtttccccacactgagtgggtggagactgaagttaggccagcttggcacttgatgtaattctccttggaatttgccctttttgagtttggatcttggttcattctcaagcctcagacagtggttcaaagtttttttcttccatttcaggtgtcgtgacaagtttgtacaaaaaagcaggctgccaccatgtcatcctcaggcacgccagacttacctgtcctactcaccgatttgaagattcaatatactaagatcttcataaacaatgaatggcatgattcagtgagtggcaagaaatttcctgtctttaatcctgcaactgaggaggagctctgccaggtagaagaaggagataaggaggatgttgacaaggcagtgaaggccgcaagacaggcttttcagattggatccccgtggcgtactatggatgcttccgagagggggcgactattatacaagttggctgatttaatcgaaagagatcgtctgctgctggcgacaatggagtcaatgaatggtggaaaactctattccaatgcatatctgaatgatttagcaggctgcatcaaaacattgcgctactgtgcaggttgggctgacaagatccagggccgtacaataccaattgatggaaatttttttacatatacaagacatgaacctattggtgtatgtggccaaatcattccttggaatttcccgttggttatgctcatttggaagatagggcctgcactgagctgtggaaacacagtggttgtcaaaccagcagagcaaactcctctcactgctctccacgtggcatctttaataaaagaggcagggtttcctcctggagtagtgaatattgttcctggttatgggcctacagcaggggcagccatttcttctcacatggatatagacaaagtagccttcacaggatcaacagaggttggcaagttgatcaaagaagctgccgggaaaagcaatctgaagagggtgaccctggagcttggaggaaagagcccttgcattgtgttagctgatgccgacttggacaatgctgttgaatttgcacaccatggggtattctaccaccagggccagtgttgtatagccgcatccaggatttttgtggaagaatcaatttatgatgagtttgttcgaaggagtgttgagcgggctaagaagtatatccttggaaatcctctgaccccaggagtcactcaaggccctcagattgacaaggaacaatatgataaaatacttgacctcattgagagtgggaagaaagaaggggccaaactggaatgtggaggaggcccgtgggggaataaaggctactttgtccagcccacagtgttctctaatgttacagatgagatgcgcattgccaaagaggagatttttggaccagtgcagcaaatcatgaagtttaaatctttagatgacgtgatcaaaagagcaaacaatactttctatggcttatcagcaggagtgtttaccaaagacattgataaagccataacaatctcctctgctctgcaggcaggaacagtgtgggtgaattgctatggcgtggtaagtgcccagtgcccctttggtggattcaagatgtctggaaatggaagagaactgggagagtacggtttccatgaatatacagaggtcaaaacagtcacagtgaaaatctctcagaagaactcaggaagcggagagggcaggggaagtcttctaacatgcggggacgtggaggaaaatcccggccccatggtgagcaagggcgaggagctgttcaccggggtggtgcccatcctggtcgagctggacggcgacgtaaacggccacaagttcagcgtgtccggcgagggcgagggcgatgccacctacggcaagctgaccctgaagttcatctgcaccaccggcaagctgcccgtgccctggcccaccctcgtgaccaccctgacctacggcgtgcagtgcttcagccgctaccccgaccacatgaagcagcacgacttcttcaagtccgccatgcccgaaggctacgtccaggagcgcaccatcttcttcaaggacgacggcaactacaagacccgcgccgaggtgaagttcgagggcgacaccctggtgaaccgcatcgagctgaagggcatcgacttcaaggaggacggcaacatcctggggcacaagctggagtacaactacaacagccacaacgtctatatcatggccgacaagcagaagaacggcatcaaggtgaacttcaagatccgccacaacatcgaggacggcagcgtgcagctcgccgaccactaccagcagaacacccccatcggcgacggccccgtgctgctgcccgacaaccactacctgagcacccagtccgccctgagcaaagaccccaacgagaagcgcgatcacatggtcctgctggagttcgtgaccgccgccgggatcactctcggcatggacgagctgtacaagtaaacccagctttcttgtacaaagtggtgataatcgaattccgataatcaacctctggattacaaaatttgtgaaagattgactggtattcttaactatgttgctccttttacgctatgtggatacgctgctttaatgcctttgtatcatgctattgcttcccgtatggctttcattttctcctccttgtataaatcctggttgctgtctctttatgaggagttgtggcccgttgtcaggcaacgtggcgtggtgtgcactgtgtttgctgacgcaacccccactggttggggcattgccaccacctgtcagctcctttccgggactttcgctttccccctccctattgccacggcggaactcatcgccgcctgccttgcccgctgctggacaggggctcggctgttgggcactgacaattccgtggtgttgtcggggaagctgacgtcctttccatggctgctcgcctgtgttgccacctggattctgcgcgggacgtccttctgctacgtcccttcggccctcaatccagcggaccttccttcccgcggcctgctgccggctctgcggcctcttccgcgtcttcgccttcgccctcagacgagtcggatctccctttgggccgcctccccgcatcgggaattcccgcggttcgaattctaccgggtaggggaggcgcttttcccaaggcagtctggagcatgcgctttagcagccccgctgggcacttggcgctacacaagtggcctctggcctcgcacacattccacatccaccggtaggcgccaaccggctccgttctttggtggccccttcgcgccaccttctactcctcccctagtcaggaagttcccccccgccccgcagctcgcgtcgtgcaggacgtgacaaatggaagtagcacgtctcactagtctcgtgcagatggacagcaccgctgagcaatggaagcgggtaggcctttggggcagcggccaatagcagctttgctccttcgctttctgggctcagaggctgggaaggggtgggtccgggggcgggctcaggggcgggctcaggggcggggcgggcgcccgaaggtcctccggaggcccggcattctgcacgcttcaaaagcgcacgtctgccgcgctgttctcctcttcctcatctccgggcctttcgacctcacgtggccaccatgaccgagtacaagcccacggtgcgcctcgccacccgcgacgacgtccccagggccgtacgcaccctcgccgccgcgttcgccgactaccccgccacgcgccacaccgtcgatccggaccgccacatcgagcgggtcaccgagctgcaagaactcttcctcacgcgcgtcgggctcgacatcggcaaggtgtgggtcgcggacgacggcgccgcggtggcggtctggaccacgccggagagcgtcgaagcgggggcggtgttcgccgagatcggcccgcgcatggccgagttgagcggttcccggctggccgcgcagcaacagatggaaggcctcctggcgccgcaccggcccaaggagcccgcgtggttcctggccaccgtcggcgtctcgcccgaccaccagggcaagggtctgggcagcgccgtcgtgctccccggagtggaggcggccgagcgcgccggggtgcccgccttcctggagacctccgcgccccgcaacctccccttctacgagcggctcggcttcaccgtcaccgccgacgtcgaggtgcccgaaggaccgcgcacctggtgcatgacccgcaagcccggtgcctgaggtacctttaagaccaatgacttacaaggcagctgtagatcttagccactttttaaaagaaaaggggggactggaagggctaattcactcccaacgaagacaagatctgctttttgcttgtactgggtctctctggttagaccagatctgagcctgggagctctctggctaactagggaacccactgcttaagcctcaataaagcttgccttgagtgcttcaagtagtgtgtgcccgtctgttgtgtgactctggtaactagagatccctcagacccttttagtcagtgtggaaaatctctagcagtagtagttcatgtcatcttattattcagtatttataacttgcaaagaaatgaatatcagagagtgagaggaacttgtttattgcagcttataatggttacaaataaagcaatagcatcacaaatttcacaaataaagcatttttttcactgcattctagttgtggtttgtccaaactcatcaatgtatcttatcatgtctggctctagctatcccgcccctaactccgcccatcccgcccctaactccgcccagttccgcccattctccgccccatggctgactaattttttttatttatgcagaggccgaggccgcctcggcctctgagctattccagaagtagtgaggaggcttttttggaggcctagggacgtacccaattcgccctatagtgagtcgtattacgcgcgctcactggccgtcgttttacaacgtcgtgactgggaaaaccctggcgttacccaacttaatcgccttgcagcacatccccctttcgccagctggcgtaatagcgaagaggcccgcaccgatcgcccttcccaacagttgcgcagcctgaatggcgaatgggacgcgccctgtagcggcgcattaagcgcggcgggtgtggtggttacgcgcagcgtgaccgctacacttgccagcgccctagcgcccgctcctttcgctttcttcccttcctttctcgccacgttcgccggctttccccgtcaagctctaaatcgggggctccctttagggttccgatttagtgctttacggcacctcgaccccaaaaaacttgattagggtgatggttcacgtagtgggccatcgccctgatagacggtttttcgccctttgacgttggagtccacgttctttaatagtggactcttgttccaaactggaacaacactcaaccctatctcggtctattcttttgatttataagggattttgccgatttcggcctattggttaaaaaatgagctgatttaacaaaaatttaacgcgaattttaacaaaatattaacgcttacaatttaggtggcacttttcggggaaatgtgcgcggaacccctatttgtttatttttctaaatacattcaaatatgtatccgctcatgagacaataaccctgataaatgcttcaataatattgaaaaaggaagagtatgagtattcaacatttccgtgtcgcccttattcccttttttgcggcattttgccttcctgtttttgctcacccagaaacgctggtgaaagtaaaagatgctgaagatcagttgggtgcacgagtgggttacatcgaactggatctcaacagcggtaagatccttgagagttttcgccccgaagaacgttttccaatgatgagcacttttaaagttctgctatgtggcgcggtattatcccgtattgacgccgggcaagagcaactcggtcgccgcatacactattctcagaatgacttggttgagtactcaccagtcacagaaaagcatcttacggatggcatgacagtaagagaattatgcagtgctgccataaccatgagtgataacactgcggccaacttacttctgacaacgatcggaggaccgaaggagctaaccgcttttttgcacaacatgggggatcatgtaactcgccttgatcgttgggaaccggagctgaatgaagccataccaaacgacgagcgtgacaccacgatgcctgtagcaatggcaacaacgttgcgcaaactattaactggcgaactacttactctagcttcccggcaacaattaatagactggatggaggcggataaagttgcaggaccacttctgcgctcggcccttccggctggctggtttattgctgataaatctggagccggtgagcgtgggtctcgcggtatcattgcagcactggggccagatggtaagccctcccgtatcgtagttatctacacgacggggagtcaggcaactatggatgaacgaaatagacagatcgctgagataggtgcctcactgattaagcattggtaactgtcagaccaagtttactcatatatactttagattgatttaaaacttcatttttaatttaaaaggatctaggtgaagatcctttttgataatctcatgaccaaaatcccttaacgtgagttttcgttccactgagcgtcagaccccgtagaaaagatcaaaggatcttcttgagatcctttttttctgcgcgtaatctgctgcttgcaaacaaaaaaaccaccgctaccagcggtggtttgtttgccggatcaagagctaccaactctttttccgaaggtaactggcttcagcagagcgcagataccaaatactgttcttctagtgtagccgtagttaggccaccacttcaagaactctgtagcaccgcctacatacctcgctctgctaatcctgttaccagtggctgctgccagtggcgataagtcgtgtcttaccgggttggactcaagacgatagttaccggataaggcgcagcggtcgggctgaacggggggttcgtgcacacagcccagcttggagcgaacgacctacaccgaactgagatacctacagcgtgagctatgagaaagcgccacgcttcccgaagagagaaaggcggacaggtatccggtaagcggcagggtcggaacaggagagcgcacgagggagcttccagggggaaacgcctggtatctttatagtcctgtcgggtttcgccacctctgacttgagcgtcgatttttgtgatgctcgtcaggggggcggagcctatggaaaaacgccagcaacgcggcctttttacggttcctggccttttgctggccttttgctcacatgttctttcctgcgttatcccctgattctgtggataaccgtattaccgcctttgagtgagctgataccgctcgccgcagccgaacgaccgagcgcagcgagtcagtgagcgaggaagcggaagagcgcccaatacgcaaaccgcctctccccgcgcgttggccgattcattaatgcagctggcacgacaggtttcccgactggaaagcgggcagtgagcgcaacgcaattaatgtgagttagctcactcattaggcaccccaggctttacactttatgcttccggctcgtatgttgtgtggaattgtgagcggataacaatttcacacaggaaacagctatgaccatgattacgccaagcgcgcaattaaccctcactaaagggaacaaaagctggagctgcaagctt

SEQ ID NO: 3 - DNA, 408 bp, Artificial Sequence
  Membrane Anchored C46 Fusion Inhibitor
atgggcgccggcgccaccggcagagccatggacggccccagactgctgctgctgctgctgctgggcgtgagcctgggcggcgccagaagctggatggagtgggacagagagatcaacaactacaccagcctgatccacagcctgatcgaggagagccagaaccagcaggagaagaacgagcaggagctgctggagctggacaagtgggccagcctgtggaactggttcagaagcgagagaaagtgctgcgtggagtgccccccctgccccgccccccccgtggccggccccctgatcgccctggtgaccagcggcgccctgctggccgtgctgggcatcaccggctacttcctgatgaacagaagaagctggagccccaccggcgagagactggagctggagccctaa

SEQ ID NO: 4 - DNA, 9623 bp, Artificial Sequence
  pLV: hALDH1A1:T2A:maC46:shCCR5
aatgtagtcttatgcaatactcttgtagtcttgcaacatggtaacgatgagttagcaacatgccttacaaggagagaaaaagcaccgtgcatgccgattggtggaagtaaggtggtacgatcgtgccttattaggaaggcaacagacgggtctgacatggattggacgaaccactgaattgccgcattgcagagatattgtatttaagtgcctagctcgatacataaacgggtctctctggttagaccagatctgagcctgggagctctctggctaactagggaacccactgcttaagcctcaataaagcttgccttgagtgcttcaagtagtgtgtgcccgtctgttgtgtgactctggtaactagagatccctcagacccttttagtcagtgtggaaaatctctagcagtggcgcccgaacagggacttgaaagcgaaagggaaaccagaggagctctctcgacgcaggactcggcttgctgaagcgcgcacggcaagaggcgaggggcggcgactggtgagtacgccaaaaattttgactagcggaggctagaaggagagagatgggtgcgagagcgtcagtattaagcgggggagaattagatcgcgatgggaaaaaattcggttaaggccagggggaaagaaaaaatataaattaaaacatatagtatgggcaagcagggagctagaacgattcgcagttaatcctggcctgttagaaacatcagaaggctgtagacaaatactgggacagctacaaccatcccttcagacaggatcagaagaacttagatcattatataatacagtagcaaccctctattgtgtgcatcaaaggatagagataaaagacaccaaggaagctttagacaagatagaggaagagcaaaacaaaagtaagaccaccgcacagcaagcggccgctgatcttcagacctggaggaggagatatgagggacaattggagaagtgaattatataaatataaagtagtaaaaattgaaccattaggagtagcacccaccaaggcaaagagaagagtggtgcagagagaaaaaagagcagtgggaataggagctttgttccttgggttcttgggagcagcaggaagcactatgggcgcagcgtcaatgacgctgacggtacaggccagacaattattgtctggtatagtgcagcagcagaacaatttgctgagggctattgaggcgcaacagcatctgttgcaactcacagtctggggcatcaagcagctccaggcaagaatcctggctgtggaaagatacctaaaggatcaacagctcctggggatttggggttgctctggaaaactcatttgcaccactgctgtgccttggaatgctagttggagtaataaatctctggaacagatttggaatcacacgacctggatggagtgggacagagaaattaacaattacacaagcttaatacactccttaattgaagaatcgcaaaaccagcaagaaaagaatgaacaagaattattggaattagataaatgggcaagtttgtggaattggtttaacataacaaattggctgtggtatataaaattattcataatgatagtaggaggcttggtaggtttaagaatagtttttgctgtactttctatagtgaatagagttaggcagggatattcaccattatcgtttcagacccacctcccaaccccgaggggacccgacaggcccgaaggaatagaagaagaaggtggagagagagacagagacagatccattcgattagtgaacggatctcgacggtatcgctagcttttaaaagaaaaggggggattggggggtacagtgcaggggaaagaatagtagacataatagcaacagacatacaaactaaagaattacaaaaacaaattacaaaaattcaaaattttactagtgattatcggatcaactttgtatagaaaagttggaattcgaacgctgacgtcatcaacccgctccaaggaatcgcgggcccagtgtcactaggcgggaacacccagcgcgcgtgcgccctggcaggaagatggctgtgagggacaggggagtggcgccctgcaatatttgcatgtcgctatgtgttctgggaaatcaccataaacgtgaaatgtctttggatttgggaatcttataagttctgtatgagaccaccgggtccatacagtcagtatcaattctcgagaattgatactgactgtatggatttttggatcccaagtttgtacaaaaaagcaggctggctccggtgcccgtcagtgggcagagcgcacatcgcccacagtccccgagaagttggggggaggggtcggcaattgaaccggtgcctagagaaggtggcgcggggtaaactgggaaagtgatgtcgtgtactggctccgcctttttcccgagggtgggggagaaccgtatataagtgcagtagtcgccgtgaacgttctttttcgcaacgggtttgccgccagaacacaggtaagtgccgtgtgtggttcccgcgggcctggcctctttacgggttatggcccttgcgtgccttgaattacttccacctggctgcagtacgtgattcttgatcccgagcttcgggttggaagtgggtgggagagttcgaggccttgcgcttaaggagccccttcgcctcgtgcttgagttgaggcctggcctgggcgctggggccgccgcgtgcgaatctggtggcaccttcgcgcctgtctcgctgctttcgataagtctctagccatttaaaatttttgatgacctgctgcgacgctttttttctggcaagatagtcttgtaaatgcgggccaagatctgcacactggtatttcggtttttggggccgcgggcggcgacggggcccgtgcgtcccagcgcacatgttcggcgaggcggggcctgcgagcgcggccaccgagaatcggacgggggtagtctcaagctggccggcctgctctggtgcctggtctcgcgccgccgtgtatcgccccgccctgggcggcaaggctggcccggtcggcaccagttgcgtgagcggaaagatggccgcttcccggccctgctgcagggagctcaaaatggaggacgcggcgctcgggagagcgggcgggtgagtcacccacacaaaggaaaagggcctttccgtcctcagccgtcgcttcatgtgactccacggagtaccgggcgccgtccaggcacctcgattagttctcgagcttttggagtacgtcgtctttaggttggggggaggggttttatgcgatggagtttccccacactgagtgggtggagactgaagttaggccagcttggcacttgatgtaattctccttggaatttgccctttttgagtttggatcttggttcattctcaagcctcagacagtggttcaaagtttttttcttccatttcaggtgtcgtgagccaccatgtcatcctcaggcacgccagacttacctgtcctactcaccgatttgaagattcaatatactaagatcttcataaacaatgaatggcatgattcagtgagtggcaagaaatttcctgtctttaatcctgcaactgaggaggagctctgccaggtagaagaaggagataaggaggatgttgacaaggcagtgaaggccgcaagacaggcttttcagattggatccccgtggcgtactatggatgcttccgagagggggcgactattatacaagttggctgatttaatcgaaagagatcgtctgctgctggcgacaatggagtcaatgaatggtggaaaactctattccaatgcatatctgaatgatttagcaggctgcatcaaaacattgcgctactgtgcaggttgggctgacaagatccagggccgtacaataccaattgatggaaatttttttacatatacaagacatgaacctattggtgtatgtggccaaatcattccttggaatttcccgttggttatgctcatttggaagatagggcctgcactgagctgtggaaacacagtggttgtcaaaccagcagagcaaactcctctcactgctctccacgtggcatctttaataaaagaggcagggtttcctcctggagtagtgaatattgttcctggttatgggcctacagcaggggcagccatttcttctcacatggatatagacaaagtagccttcacaggatcaacagaggttggcaagttgatcaaagaagctgccgggaaaagcaatctgaagagggtgaccctggagcttggaggaaagagcccttgcattgtgttagctgatgccgacttggacaatgctgttgaatttgcacaccatggggtattctaccaccagggccagtgttgtatagccgcatccaggatttttgtggaagaatcaatttatgatgagtttgttcgaaggagtgttgagcgggctaagaagtatatccttggaaatcctctgaccccaggagtcactcaaggccctcagattgacaaggaacaatatgataaaatacttgacctcattgagagtgggaagaaagaaggggccaaactggaatgtggaggaggcccgtgggggaataaaggctactttgtccagcccacagtgttctctaatgttacagatgagatgcgcattgccaaagaggagatttttggaccagtgcagcaaatcatgaagtttaaatctttagatgacgtgatcaaaagagcaaacaatactttctatggcttatcagcaggagtgtttaccaaagacattgataaagccataacaatctcctctgctctgcaggcaggaacagtgtgggtgaattgctatggcgtggtaagtgcccagtgcccctttggtggattcaagatgtctggaaatggaagagaactgggagagtacggtttccatgaatatacagaggtcaaaacagtcacagtgaaaatctctcagaagaactcaggaagcggagagggcaggggaagtcttctaacatgcggggacgtggaggaaaatcccggccccatgggcgccggcgccaccggcagagccatggacggccccagactgctgctgctgctgctgctgggcgtgagcctgggcggcgccagaagctggatggagtgggacagagagatcaacaactacaccagcctgatccacagcctgatcgaggagagccagaaccagcaggagaagaacgagcaggagctgctggagctggacaagtgggccagcctgtggaactggttcagaagcgagagaaagtgctgcgtggagtgccccccctgccccgccccccccgtggccggccccctgatcgccctggtgaccagcggcgccctgctggccgtgctgggcatcaccggctacttcctgatgaacagaagaagctggagccccaccggcgagagactggagctggagccctaaacccagctttcttgtacaaagtggtgataatcgaattccgataatcaacctctggattacaaaatttgtgaaagattgactggtattcttaactatgttgctccttttacgctatgtggatacgctgctttaatgcctttgtatcatgctattgcttcccgtatggctttcattttctcctccttgtataaatcctggttgctgtctctttatgaggagttgtggcccgttgtcaggcaacgtggcgtggtgtgcactgtgtttgctgacgcaacccccactggttggggcattgccaccacctgtcagctcctttccgggactttcgctttccccctccctattgccacggcggaactcatcgccgcctgccttgcccgctgctggacaggggctcggctgttgggcactgacaattccgtggtgttgtcggggaagctgacgtcctttccatggctgctcgcctgtgttgccacctggattctgcgcgggacgtccttctgctacgtcccttcggccctcaatccagcggaccttccttcccgcggcctgctgccggctctgcggcctcttccgcgtcttcgccttcgccctcagacgagtcggatctccctttgggccgcctccccgcatcgggaattcccgcggttcgctttaagaccaatgacttacaaggcagctgtagatcttagccactttttaaaagaaaaggggggactggaagggctaattcactcccaacgaagacaagatctgctttttgcttgtactgggtctctctggttagaccagatctgagcctgggagctctctggctaactagggaacccactgcttaagcctcaataaagcttgccttgagtgcttcaagtagtgtgtgcccgtctgttgtgtgactctggtaactagagatccctcagacccttttagtcagtgtggaaaatctctagcagtagtagttcatgtcatcttattattcagtatttataacttgcaaagaaatgaatatcagagagtgagaggaacttgtttattgcagcttataatggttacaaataaagcaatagcatcacaaatttcacaaataaagcatttttttcactgcattctagttgtggtttgtccaaactcatcaatgtatcttatcatgtctggctctagctatcccgcccctaactccgcccatcccgcccctaactccgcccagttccgcccattctccgccccatggctgactaattttttttatttatgcagaggccgaggccgcctcggcctctgagctattccagaagtagtgaggaggcttttttggaggcctagggacgtacccaattcgccctatagtgagtcgtattacgcgcgctcactggccgtcgttttacaacgtcgtgactgggaaaaccctggcgttacccaacttaatcgccttgcagcacatccccctttcgccagctggcgtaatagcgaagaggcccgcaccgatcgcccttcccaacagttgcgcagcctgaatggcgaatgggacgcgccctgtagcggcgcattaagcgcggcgggtgtggtggttacgcgcagcgtgaccgctacacttgccagcgccctagcgcccgctcctttcgctttcttcccttcctttctcgccacgttcgccggctttccccgtcaagctctaaatcgggggctccctttagggttccgatttagtgctttacggcacctcgaccccaaaaaacttgattagggtgatggttcacgtagtgggccatcgccctgatagacggtttttcgccctttgacgttggagtccacgttctttaatagtggactcttgttccaaactggaacaacactcaaccctatctcggtctattcttttgatttataagggattttgccgatttcggcctattggttaaaaaatgagctgatttaacaaaaatttaacgcgaattttaacaaaatattaacgcttacaatttaggtggcacttttcggggaaatgtgcgcggaacccctatttgtttatttttctaaatacattcaaatatgtatccgctcatgagacaataaccctgataaatgcttcaataatattgaaaaaggaagagtatgagtattcaacatttccgtgtcgcccttattcccttttttgcggcattttgccttcctgtttttgctcacccagaaacgctggtgaaagtaaaagatgctgaagatcagttgggtgcacgagtgggttacatcgaactggatctcaacagcggtaagatccttgagagttttcgccccgaagaacgttttccaatgatgagcacttttaaagttctgctatgtggcgcggtattatcccgtattgacgccgggcaagagcaactcggtcgccgcatacactattctcagaatgacttggttgagtactcaccagtcacagaaaagcatcttacggatggcatgacagtaagagaattatgcagtgctgccataaccatgagtgataacactgcggccaacttacttctgacaacgatcggaggaccgaaggagctaaccgcttttttgcacaacatgggggatcatgtaactcgccttgatcgttgggaaccggagctgaatgaagccataccaaacgacgagcgtgacaccacgatgcctgtagcaatggcaacaacgttgcgcaaactattaactggcgaactacttactctagcttcccggcaacaattaatagactggatggaggcggataaagttgcaggaccacttctgcgctcggcccttccggctggctggtttattgctgataaatctggagccggtgagcgtgggtctcgcggtatcattgcagcactggggccagatggtaagccctcccgtatcgtagttatctacacgacggggagtcaggcaactatggatgaacgaaatagacagatcgctgagataggtgcctcactgattaagcattggtaactgtcagaccaagtttactcatatatactttagattgatttaaaacttcatttttaatttaaaaggatctaggtgaagatcctttttgataatctcatgaccaaaatcccttaacgtgagttttcgttccactgagcgtcagaccccgtagaaaagatcaaaggatcttcttgagatcctttttttctgcgcgtaatctgctgcttgcaaacaaaaaaaccaccgctaccagcggtggtttgtttgccggatcaagagctaccaactctttttccgaaggtaactggcttcagcagagcgcagataccaaatactgttcttctagtgtagccgtagttaggccaccacttcaagaactctgtagcaccgcctacatacctcgctctgctaatcctgttaccagtggctgctgccagtggcgataagtcgtgtcttaccgggttggactcaagacgatagttaccggataaggcgcagcggtcgggctgaacggggggttcgtgcacacagcccagcttggagcgaacgacctacaccgaactgagatacctacagcgtgagctatgagaaagcgccacgcttcccgaagagagaaaggcggacaggtatccggtaagcggcagggtcggaacaggagagcgcacgagggagcttccagggggaaacgcctggtatctttatagtcctgtcgggtttcgccacctctgacttgagcgtcgatttttgtgatgctcgtcaggggggcggagcctatggaaaaacgccagcaacgcggcctttttacggttcctggccttttgctggccttttgctcacatgttctttcctgcgttatcccctgattctgtggataaccgtattaccgcctttgagtgagctgataccgctcgccgcagccgaacgaccgagcgcagcgagtcagtgagcgaggaagcggaagagcgcccaatacgcaaaccgcctctccccgcgcgttggccgattcattaatgcagctggcacgacaggtttcccgactggaaagcgggcagtgagcgcaacgcaattaatgtgagttagctcactcattaggcaccccaggctttacactttatgcttccggctcgtatgttgtgtggaattgtgagcggataacaatttcacacaggaaacagctatgaccatgattacgccaagcgcgcaattaaccctcactaaagggaacaaaagctggagctgcaagctt

SEQ ID NO: 5 - DNA, 8059 bp, Artificial Sequence
  pLV: maC46:shCCR5
aatgtagtcttatgcaatactcttgtagtcttgcaacatggtaacgatgagttagcaacatgccttacaaggagagaaaaagcaccgtgcatgccgattggtggaagtaaggtggtacgatcgtgccttattaggaaggcaacagacgggtctgacatggattggacgaaccactgaattgccgcattgcagagatattgtatttaagtgcctagctcgatacataaacgggtctctctggttagaccagatctgagcctgggagctctctggctaactagggaacccactgcttaagcctcaataaagcttgccttgagtgcttcaagtagtgtgtgcccgtctgttgtgtgactctggtaactagagatccctcagacccttttagtcagtgtggaaaatctctagcagtggcgcccgaacagggacttgaaagcgaaagggaaaccagaggagctctctcgacgcaggactcggcttgctgaagcgcgcacggcaagaggcgaggggcggcgactggtgagtacgccaaaaattttgactagcggaggctagaaggagagagatgggtgcgagagcgtcagtattaagcgggggagaattagatcgcgatgggaaaaaattcggttaaggccagggggaaagaaaaaatataaattaaaacatatagtatgggcaagcagggagctagaacgattcgcagttaatcctggcctgttagaaacatcagaaggctgtagacaaatactgggacagctacaaccatcccttcagacaggatcagaagaacttagatcattatataatacagtagcaaccctctattgtgtgcatcaaaggatagagataaaagacaccaaggaagctttagacaagatagaggaagagcaaaacaaaagtaagaccaccgcacagcaagcggccgctgatcttcagacctggaggaggagatatgagggacaattggagaagtgaattatataaatataaagtagtaaaaattgaaccattaggagtagcacccaccaaggcaaagagaagagtggtgcagagagaaaaaagagcagtgggaataggagctttgttccttgggttcttgggagcagcaggaagcactatgggcgcagcgtcaatgacgctgacggtacaggccagacaattattgtctggtatagtgcagcagcagaacaatttgctgagggctattgaggcgcaacagcatctgttgcaactcacagtctggggcatcaagcagctccaggcaagaatcctggctgtggaaagatacctaaaggatcaacagctcctggggatttggggttgctctggaaaactcatttgcaccactgctgtgccttggaatgctagttggagtaataaatctctggaacagatttggaatcacacgacctggatggagtgggacagagaaattaacaattacacaagcttaatacactccttaattgaagaatcgcaaaaccagcaagaaaagaatgaacaagaattattggaattagataaatgggcaagtttgtggaattggtttaacataacaaattggctgtggtatataaaattattcataatgatagtaggaggcttggtaggtttaagaatagtttttgctgtactttctatagtgaatagagttaggcagggatattcaccattatcgtttcagacccacctcccaaccccgaggggacccgacaggcccgaaggaatagaagaagaaggtggagagagagacagagacagatccattcgattagtgaacggatctcgacggtatcgctagcttttaaaagaaaaggggggattggggggtacagtgcaggggaaagaatagtagacataatagcaacagacatacaaactaaagaattacaaaaacaaattacaaaaattcaaaattttactagtgattatcggatcaactttgtatagaaaagttggaattcgaacgctgacgtcatcaacccgctccaaggaatcgcgggcccagtgtcactaggcgggaacacccagcgcgcgtgcgccctggcaggaagatggctgtgagggacaggggagtggcgccctgcaatatttgcatgtcgctatgtgttctgggaaatcaccataaacgtgaaatgtctttggatttgggaatcttataagttctgtatgagaccaccgggtccatacagtcagtatcaattctcgagaattgatactgactgtatggatttttggatcccaagtttgtacaaaaaagcaggctggctccggtgcccgtcagtgggcagagcgcacatcgcccacagtccccgagaagttggggggaggggtcggcaattgaaccggtgcctagagaaggtggcgcggggtaaactgggaaagtgatgtcgtgtactggctccgcctttttcccgagggtgggggagaaccgtatataagtgcagtagtcgccgtgaacgttctttttcgcaacgggtttgccgccagaacacaggtaagtgccgtgtgtggttcccgcgggcctggcctctttacgggttatggcccttgcgtgccttgaattacttccacctggctgcagtacgtgattcttgatcccgagcttcgggttggaagtgggtgggagagttcgaggccttgcgcttaaggagccccttcgcctcgtgcttgagttgaggcctggcctgggcgctggggccgccgcgtgcgaatctggtggcaccttcgcgcctgtctcgctgctttcgataagtctctagccatttaaaatttttgatgacctgctgcgacgctttttttctggcaagatagtcttgtaaatgcgggccaagatctgcacactggtatttcggtttttggggccgcgggcggcgacggggcccgtgcgtcccagcgcacatgttcggcgaggcggggcctgcgagcgcggccaccgagaatcggacgggggtagtctcaagctggccggcctgctctggtgcctggtctcgcgccgccgtgtatcgccccgccctgggcggcaaggctggcccggtcggcaccagttgcgtgagcggaaagatggccgcttcccggccctgctgcagggagctcaaaatggaggacgcggcgctcgggagagcgggcgggtgagtcacccacacaaaggaaaagggcctttccgtcctcagccgtcgcttcatgtgactccacggagtaccgggcgccgtccaggcacctcgattagttctcgagcttttggagtacgtcgtctttaggttggggggaggggttttatgcgatggagtttccccacactgagtgggtggagactgaagttaggccagcttggcacttgatgtaattctccttggaatttgccctttttgagtttggatcttggttcattctcaagcctcagacagtggttcaaagtttttttcttccatttcaggtgtcgtgagccaccatgggcgccggcgccaccggcagagccatggacggccccagactgctgctgctgctgctgctgggcgtgagcctgggcggcgccagaagctggatggagtgggacagagagatcaacaactacaccagcctgatccacagcctgatcgaggagagccagaaccagcaggagaagaacgagcaggagctgctggagctggacaagtgggccagcctgtggaactggttcagaagcgagagaaagtgctgcgtggagtgccccccctgccccgccccccccgtggccggccccctgatcgccctggtgaccagcggcgccctgctggccgtgctgggcatcaccggctacttcctgatgaacagaagaagctggagccccaccggcgagagactggagctggagccctaaaaacccagctttcttgtacaaagtggtgataatcgaattccgataatcaacctctggattacaaaatttgtgaaagattgactggtattcttaactatgttgctccttttacgctatgtggatacgctgctttaatgcctttgtatcatgctattgcttcccgtatggctttcattttctcctccttgtataaatcctggttgctgtctctttatgaggagttgtggcccgttgtcaggcaacgtggcgtggtgtgcactgtgtttgctgacgcaacccccactggttggggcattgccaccacctgtcagctcctttccgggactttcgctttccccctccctattgccacggcggaactcatcgccgcctgccttgcccgctgctggacaggggctcggctgttgggcactgacaattccgtggtgttgtcggggaagctgacgtcctttccatggctgctcgcctgtgttgccacctggattctgcgcgggacgtccttctgctacgtcccttcggccctcaatccagcggaccttccttcccgcggcctgctgccggctctgcggcctcttccgcgtcttcgccttcgccctcagacgagtcggatctccctttgggccgcctccccgcatcgggaattcccgcggttcgctttaagaccaatgacttacaaggcagctgtagatcttagccactttttaaaagaaaaggggggactggaagggctaattcactcccaacgaagacaagatctgctttttgcttgtactgggtctctctggttagaccagatctgagcctgggagctctctggctaactagggaacccactgcttaagcctcaataaagcttgccttgagtgcttcaagtagtgtgtgcccgtctgttgtgtgactctggtaactagagatccctcagacccttttagtcagtgtggaaaatctctagcagtagtagttcatgtcatcttattattcagtatttataacttgcaaagaaatgaatatcagagagtgagaggaacttgtttattgcagcttataatggttacaaataaagcaatagcatcacaaatttcacaaataaagcatttttttcactgcattctagttgtggtttgtccaaactcatcaatgtatcttatcatgtctggctctagctatcccgcccctaactccgcccatcccgcccctaactccgcccagttccgcccattctccgccccatggctgactaattttttttatttatgcagaggccgaggccgcctcggcctctgagctattccagaagtagtgaggaggcttttttggaggcctagggacgtacccaattcgccctatagtgagtcgtattacgcgcgctcactggccgtcgttttacaacgtcgtgactgggaaaaccctggcgttacccaacttaatcgccttgcagcacatccccctttcgccagctggcgtaatagcgaagaggcccgcaccgatcgcccttcccaacagttgcgcagcctgaatggcgaatgggacgcgccctgtagcggcgcattaagcgcggcgggtgtggtggttacgcgcagcgtgaccgctacacttgccagcgccctagcgcccgctcctttcgctttcttcccttcctttctcgccacgttcgccggctttccccgtcaagctctaaatcgggggctccctttagggttccgatttagtgctttacggcacctcgaccccaaaaaacttgattagggtgatggttcacgtagtgggccatcgccctgatagacggtttttcgccctttgacgttggagtccacgttctttaatagtggactcttgttccaaactggaacaacactcaaccctatctcggtctattcttttgatttataagggattttgccgatttcggcctattggttaaaaaatgagctgatttaacaaaaatttaacgcgaattttaacaaaatattaacgcttacaatttaggtggcacttttcggggaaatgtgcgcggaacccctatttgtttatttttctaaatacattcaaatatgtatccgctcatgagacaataaccctgataaatgcttcaataatattgaaaaaggaagagtatgagtattcaacatttccgtgtcgcccttattcccttttttgcggcattttgccttcctgtttttgctcacccagaaacgctggtgaaagtaaaagatgctgaagatcagttgggtgcacgagtgggttacatcgaactggatctcaacagcggtaagatccttgagagttttcgccccgaagaacgttttccaatgatgagcacttttaaagttctgctatgtggcgcggtattatcccgtattgacgccgggcaagagcaactcggtcgccgcatacactattctcagaatgacttggttgagtactcaccagtcacagaaaagcatcttacggatggcatgacagtaagagaattatgcagtgctgccataaccatgagtgataacactgcggccaacttacttctgacaacgatcggaggaccgaaggagctaaccgcttttttgcacaacatgggggatcatgtaactcgccttgatcgttgggaaccggagctgaatgaagccataccaaacgacgagcgtgacaccacgatgcctgtagcaatggcaacaacgttgcgcaaactattaactggcgaactacttactctagcttcccggcaacaattaatagactggatggaggcggataaagttgcaggaccacttctgcgctcggcccttccggctggctggtttattgctgataaatctggagccggtgagcgtgggtctcgcggtatcattgcagcactggggccagatggtaagccctcccgtatcgtagttatctacacgacggggagtcaggcaactatggatgaacgaaatagacagatcgctgagataggtgcctcactgattaagcattggtaactgtcagaccaagtttactcatatatactttagattgatttaaaacttcatttttaatttaaaaggatctaggtgaagatcctttttgataatctcatgaccaaaatcccttaacgtgagttttcgttccactgagcgtcagaccccgtagaaaagatcaaaggatcttcttgagatcctttttttctgcgcgtaatctgctgcttgcaaacaaaaaaaccaccgctaccagcggtggtttgtttgccggatcaagagctaccaactctttttccgaaggtaactggcttcagcagagcgcagataccaaatactgttcttctagtgtagccgtagttaggccaccacttcaagaactctgtagcaccgcctacatacctcgctctgctaatcctgttaccagtggctgctgccagtggcgataagtcgtgtcttaccgggttggactcaagacgatagttaccggataaggcgcagcggtcgggctgaacggggggttcgtgcacacagcccagcttggagcgaacgacctacaccgaactgagatacctacagcgtgagctatgagaaagcgccacgcttcccgaagagagaaaggcggacaggtatccggtaagcggcagggtcggaacaggagagcgcacgagggagcttccagggggaaacgcctggtatctttatagtcctgtcgggtttcgccacctctgacttgagcgtcgatttttgtgatgctcgtcaggggggcggagcctatggaaaaacgccagcaacgcggcctttttacggttcctggccttttgctggccttttgctcacatgttctttcctgcgttatcccctgattctgtggataaccgtattaccgcctttgagtgagctgataccgctcgccgcagccgaacgaccgagcgcagcgagtcagtgagcgaggaagcggaagagcgcccaatacgcaaaccgcctctccccgcgcgttggccgattcattaatgcagctggcacgacaggtttcccgactggaaagcgggcagtgagcgcaacgcaattaatgtgagttagctcactcattaggcaccccaggctttacactttatgcttccggctcgtatgttgtgtggaattgtgagcggataacaatttcacacaggaaacagctatgaccatgattacgccaagcgcgcaattaaccctcactaaagggaacaaaagctggagctgcaagctt

SEQ ID NO: 6 - DNA, 21 bp, Artificial Sequence
  hCCR5 shRNA sense
actcttgacagggctctattt

SEQ ID NO: 7 - DNA, 21 bp, Artificial Sequence
  hCCR5 shRNA antisense
aaatagagccctgtcaagagt

SEQ ID NO: 8 - DNA, 1096 bp, Artificial Sequence
  Human CD4 Promoter:-1076 to +20
aagacaggttctcactctgtcactcaggctagagtgcagtggtgcaatcacggttcactgcagcctcaacttcctgggctcaagcgatccccccacctcggcctcctaaaatgctgggattataggcatgagccaccactcccagccccacttttttcagactggaaaacgcacactcacatgtgcatctttaaatgatcacttgggctgtggtatggagaatggcgaccagtgaggaggcaggagctgttgtccgagcaagggatgatattggcatcttggattggcatggtggcagtagtggtagtgcagagtgacttgggtagattttggagccatttagaaggtaacatccacaggaactggtaaataaatacgtgggagaagttgggtgaagggggtgtcaaagattacacccaatttattttgcttgggcaagttggtggatggtgagcccctcactgagtgagaagcctggagaagcaggtttggagggtggtagtatgcaggtggtatgcatagttggggatgtgtgttgagtttgctatgtccggtgagcttcccagtggagatgtccaatgggcagacggatactcacatagagagttcatggtagattcgggctagaggaaagcacctgaggcctggccagagacgcctagaggaacagagcctggttaacagtcactcctggtgtctcagatattctctgctcagcccacgccctctcttccacactgggccacctataaagcctccacagatacccctggggcacccactggacacatgccctcagggccccagagcaaggagctgtttgtgggcttaccactgctgttcccatatgcccccaactgcctcccacttctttccccacagcctggtcagacatggcgctaccactaatggaatctttcttgccatctttttcttgccgcttaacagtggcagtgacagtttgactcctgatttaagcctgattctgcttaactttttcccttgactttggcattttcactttgacatgttccctgagagcctggggggtggggaacccagctccagctggtgacgtttggggccggcccaggcc

SEQ ID NO: 9 - DNA, 320 bp, Artificial Sequence
  Human CD3E
aaggtacggaagaggacggtggcggtggaagccgggcttggagatgggacacagatttccacaagctgcctggaaaagctgcgagccagggctggggaagtgaaggagggaggtgtctcaagcaggcacacccccaccctgaggcagccgcctgcagccagaggcgggctgtggttaagcagcgcaggatgtgggctgcactgctaagcgtggcttctgggagtgagggtgggagaggtacagcggcagctggcggaggcccgtgtgagagcgctttgttctcagtctcccacagcacactctgcttgcagagggggatc

SEQ ID NO: 10 - protein, 501 aa, Artificial Sequence
  hALDH1 protein
MSSSGTPDLPVLLTDLKIQYTKIFINNEWHDSVSGKKFPVFNPATEEELCQVEEGDKEDVDKAVKAARQAFQIGSPWRTMDASERGRLLYKLADLIERDRLLLATMESMNGGKLYSNAYLNDLAGCIKTLRYCAGWADKIQGRTIPIDGNFFTYTRHEPIGVCGQIIPWNFPLVMLIWKIGPALSCGNTVVVKPAEQTPLTALHVASLIKEAGFPPGVVNIVPGYGPTAGAAISSHMDIDKVAFTGSTEVGKLIKEAAGKSNLKRVTLELGGKSPCIVLADADLDNAVEFAHHGVFYHQGQCCIAASRIFVEESIYDEFVRRSVERAKKYILGNPLTPGVTQGPQIDKEQYDKILDLIESGKKEGAKLECGGGPWGNKGYFVQPTVFSNVTDEMRIAKEEIFGPVQQIMKFKSLDDVIKRANNTFYGLSAGVFTKDIDKAITISSALQAGTVWVNCYGVVSAQCPFGGFKMSGNGRELGEYGFHEYTEVKTVTVKISQKNS

SEQ ID NO: 11 - protein, 135 aa, Artificial Sequence [sequence omitted]

SEQ ID NO: 12 - DNA, 540 bp, Artificial Sequence
  synthetic sequence
aggatgatggtgatggggaactaaatggggaaatatggaaggtcacaggaaaagttaacacaagttagcaaaaagttaacataacacaaaaaggtcttgcaggaaaaaaaaaagaaaagaaaagaaagaaaaagtctccaagaatggtttggacagccaaaatgaatacttatagtcacgtatacctgctcactcctgacgcttcactcacacacagcacaggatctggtgaggctatcactaaatgtgccacattgtggttaagttttacctgattaacgaaatgctcacacttctaaactgaggtccttacagtagattccttttgcaagattgttactggcttacaacttaaaaataaaggaaaatcacaaggaaagaaaagtggggaaaaaatcggaggaaacttgcccctgccctggccaccggcaaggctgccacaaaggggttaaaagttaagtggaagtggagcttgaagaagtgggatggggcctctccaggaaagctgaacgaggcatctggagcccgaacaaacctcca

SEQ ID NO: 13 - DNA, 321 bp, Artificial Sequence
  synthetic sequence
tgtttgaatgaggcttcagtactttacagaatcgttgcctgcacatcttggaaacacttgctgggattacttcgacttcttaacccaacagaaggctcgagaaggtatattgctgttgacagtgagcgcactcttgacagggctctattttagtgaagccacagatgtaaaatagagccctgtcaagagtttgcctactgcctcggacttcaaggggctagaattcgagcaattatcttgtttactaaaactgaataccttgctatctctttgatacatttttacaaagctgaattaaaatggtataaattaaatcacttt

SEQ ID NO: 14 - DNA, 132 bp, Artificial Sequence
  synthetic sequence
gcctggaaggacctggagctgctggagcaggagaacaaggagcagcagaaccagagcgaggagatcctgagccacatcctgagcacctacaacaacatcgagagagactgggagatgtggaccatgaacaac

SEQ ID NO: 15 - protein, 44 aa, Artificial Sequence
  synthetic sequence
AWKDLELLEQENKEQQNQSEEILSHILSTYNNIERDWEMWTMNN

SEQ ID NO: 16 - DNA, 273 bp, Artificial Sequence
  synthetic sequence
gagctgaagacccccctgggcgacaccacccacacctgccccagatgccccgagcccaagagctgcgacaccccccccccctgccccagatgccccgagcccaagagctgcgacaccccccccccctgccccagatgccccgagcccaagagctgcgacaccccccccccctgccccagatgcccccttgaaaatggtgggacatccttatcagagaaaacagttcttctgctggtgactccatttctggcagcagcctggagccttcatccc

SEQ ID NO: 17 - protein, 91 aa, Artificial Sequence
  synthetic sequence
ELKTPLGDTTHTCPRCPEPKSCDTPPPCPRCPEPKSCDTPPPCPRCPEPKSCDTPPPCPRCPLENGGTSLSEKTVLLLVTPFLAAAWSLHP

SEQ ID NO: 18 - DNA, 405 bp, Artificial Sequence
  synthetic sequence
gcctggaaggacctggagctgctggagcaggagaacaaggagcagcagaaccagagcgaggagatcctgagccacatcctgagcacctacaacaacatcgagagagactgggagatgtggaccatgaacaacgagctgaagacccccctgggcgacaccacccacacctgccccagatgccccgagcccaagagctgcgacaccccccccccctgccccagatgccccgagcccaagagctgcgacaccccccccccctgccccagatgccccgagcccaagagctgcgacaccccccccccctgccccagatgcccccttgaaaatggtgggacatccttatcagagaaaacagttcttctgctggtgactccatttctggcagcagcctggagccttcatccc

SEQ ID NO: 19 - protein, 135 aa, Artificial Sequence
  synthetic sequence
AWKDLELLEQENKEQQNQSEEILSHILSTYNNIERDWEMWTMNNELKTPLGDTTHTCPRCPEPKSCDTPPPCPRCPEPKSCDTPPPCPRCPEPKSCDTPPPCPRCPLENGGTSLSEKTVLLLVTPFLAAAWSLHP